European Patent Application EP 4 603 592 A1, published August 20, 2025. Title: METHOD FOR GENERATING PROBES ON CARRIER AND METHOD FOR DETECTING TARGET SUBSTANCE IN SAMPLE. Applicant: SHENZHEN SALUS BIOMED CO., LTD. Application CN PCT/CN2023/124273, filed October 12, 2023. The sequence listing filed with the application follows.

SEQUENCE LISTING (7 sequences)

SEQ ID NO: 1 - DNA, 34 bp, synthetic construct
  source 1..34: mol_type = other DNA
ttttttttttcaagcagaagacggcatacgagat

SEQ ID NO: 2 - DNA, 39 bp, synthetic construct
  source 1..39: mol_type = other DNA
ttttttttttaatgatacggcgaccaccgagatctacac

SEQ ID NO: 3 - DNA, 32 bp, synthetic construct
  source 1..32: mol_type = other DNA
tcagacgtgtgctcttccgatctnnnnnnnnn

SEQ ID NO: 4 - DNA, 20 bp, synthetic construct
  source 1..20: mol_type = other DNA
tctttccctacacgacgctc

SEQ ID NO: 5 - DNA, 20 bp, synthetic construct
  source 1..20: mol_type = other DNA
tcagacgtgtgctcttccga

SEQ ID NO: 6 - DNA, 52 bp, synthetic construct
  source 1..52: mol_type = other DNA
aatgatacggcgaccaccgagatctacactctttccctacacgacgctcttc

SEQ ID NO: 7 - DNA, 55 bp, synthetic construct
  source 1..55: mol_type = other DNA
caagcagaagacggcatacgagatgtgactggagttcagacgtgtgctcttccga